European Patent Specification EP 3 502 686 B1, published November 22, 2023. Title: Antigennachweis von Trichinella. Applicant: Euroimmun Medizinische Labordiagnostika AG. The sequence listing filed with the application follows.

SEQUENCE LISTING (6 sequences)

SEQ ID NO: 1 - protein, 120 aa, Artificial Sequence
  Anti-[TRISP][B7] VH
AVTLDESGGGLQTPRGGLSLVCKASGYTFSSHNMAWVRQAPGKGLEFVAGISNTGSFTLYGAAVKGRATISRDNGQSTVRLQLNNLRAEDTGTYYCAKHAGVGLYSIDAWGHGTEVIVSS

SEQ ID NO: 2 - protein, 103 aa, Artificial Sequence
  Anti-[TRISP][B7] VL
ALTQPSSVSANLGGTVKITCSGGTSDYGWYQQKAPGSAPVTLIYDNTNRPSDIPSRFSGSLSGSTNTLTITGVQAEDEAVYFCGSADRTYAGVFGAGTTLTVL

SEQ ID NO: 3 - protein, 117 aa, Artificial Sequence
  ANTI-[TRISP][C9] VH
AVTLDESGGGLQTPGGALSLVCKASGFSISSYSMQWVRQAPGKGLEWVAGIYYDGNTWYAPAVKGRATISRDNGQSTVRLRLNNLRAEDTATYFCAKYAGGYSIDAWGHGTEVIVSS

SEQ ID NO: 4 - protein, 104 aa, Artificial Sequence
  ANTI-[TRISP][C9] VL
ALTQPSSVSANPGETVKITCSGSSGSYGWYQQKSPGSGPVTVIYYNDKRPSDIPSRFSGSASGSTATLTITGVQAEDEAVYFCGGYDSSTYVGIFGAGTTLTVL

SEQ ID NO: 5 - protein, 122 aa, Artificial Sequence
  ANTI-[TRISP][18H1] VH
QVQLKESGPGLVQPSQTLSLTCTVSGLSLTSNSVGWIRQPPGKGLEWMGIIWSNGGTDYNSAIKSRLSISRDTSKSQVFLKMHSLQTEDTAMYFCARGPYYGSYRLGYFDYWGQGVMVTVSS

SEQ ID NO: 6 - protein, 113 aa, Artificial Sequence
  ANTI-[TRISP][18H1] VL
DVVMTQSPSSLAVSAGETVTLNCQSSQSLLYSGTQNNYLAWYQQKPGQSPKLLISWASTRQSGVPLRFIGSGSGTDFTLTITSVQAEDLAIYYCQQFYDTPLTFGSGTKLEIK